European Patent Application EP 4 273 226 A1, published November 8, 2023. Title: Recombinant strain with Modified Gene BBD29_09525 for Producing L-Glutamic Acid, and Method for Constructing the Same and Use Thereof. Applicant: INNER MONGOLIA EPPEN BIOTECH CO., LTD. The sequence listing filed with the application follows.

SEQUENCE LISTING (33 sequences)

SEQ ID NO: 1 - DNA, 1503 bp, Corynebacterium glutamicum
  CDS (1)..(1503)
atgtcagattccccgaagaacgcaccgaggattaccgatgaggcagatgtagttctcattggtgccggtatcatgagctccacgctgggtgcaatgctgcgtcagctggagccaagctggactcagatcgtcttcgagcgtttggatggaccggcacaagagtcgtcctccccgtggaacaatgcaggaaccggccactctgctctatgcgagctgaactacaccccagaggttaagggcaaggttgaaattgccaaggctgtaggaatcaacgagaagttccaggtttcccgtcagttctggtctcacctcgttgaagagggcgtgctggctgatcctaaggaattcatcaaccctgttcctcacgtatctttcggccagggcgcagaccaggttgcatacatcaaggctcgctacgaagctttgaaggatcacccactcttccagggcatgacctacgctgacgatgaagctaccttcaccgagaagctgcctttgatggcaaagggccgtgacttctctgatccagtagcaatctcttggatcgatgaaggcaccgacatcaactacggtgctcagaccaagcagtacctggatgcatctgaagttgaaggcactgaaatccgctatggccacgaagtcaagagcatcaaggctgatggcgcaaagtggatcgtgaccgtcaagaacgtacacactggcgacaccaagaccatcaaggcaaacttcgtgttcgtcggcgcaggcgggtacgcactggatctgcttcgcagcgcaggcatcccacaggtcaagggcttcgctggattcccagtatccggcctgtggcttcgttgcaccaacgaggaactgatcgagcagcacgcagccaaggtatatggcaaggcatctgttggcgctcctccaatgtctgttcctcaccttgacacccgcgttatcgagggtgaaaagggtctgctctttggaccttacggtggctggacccctaagttcttgaaggaaggctcctacctggacctgttcaagtccatccgcccagacaacattccttcctaccttggcgttgctgctcaggaatttgatctgaccaagtaccttgtcactgaagttctcaaggaccaggacaagcgtatggatgctcttcgcgagtacatgccagaggcacaaaacggcgattgggagaccatcgttgccggacagcgtgttcaggttattaagcctgcaggattccctaagttcggttccctggaattcggcaccaccttgatcaacaactccgaaggcaccatcgccggattgctcggtgcttcccctggagcatccatcgcaccttccgcaatgatcgagctgcttgagcgttgcttcggtgaccgcatgatcgagtggggcgacaagctgaaggacatgatcccttcctacggcaagaagcttgcttccgagccagcactgtttgagcagcagtgggcacgcacccagaagaccctgaagcttgaggaagcctaa

SEQ ID NO: 2 - DNA, 1503 bp, Artificial Sequence
  Synthesized
  CDS (1)..(1503)
atgtcagattccccgaagaacgcaccgaggattaccgatgaggcagatgtagttctcattggtgccggtatcatgagctccacgctgggtgcaatgctgcgtcagctggagccaagctggactcagatcgtcttcgagcgtttggatggaccggcacaagagtcgtcctccccgtggaacaatgcaggaaccggccactctgctctatgcgagctgaactacaccccagaggttaagggcaaggttgaaattgccaaggctgtaggaatcaacgagaagttccaggtttcccgtcagttctggtctcacctcgttgaagagggcgtgctggctgattctaaggaattcatcaaccctgttcctcacgtatctttcggccagggcgcagaccaggttgcatacatcaaggctcgctacgaagctttgaaggatcacccactcttccagggcatgacctacgctgacgatgaagctaccttcaccgagaagctgcctttgatggcaaagggccgtgacttctctgatccagtagcaatctcttggatcgatgaaggcaccgacatcaactacggtgctcagaccaagcagtacctggatgcatctgaagttgaaggcactgaaatccgctatggccacgaagtcaagagcatcaaggctgatggcgcaaagtggatcgtgaccgtcaagaacgtacacactggcgacaccaagaccatcaaggcaaacttcgtgttcgtcggcgcaggcgggtacgcactggatctgcttcgcagcgcaggcatcccacaggtcaagggcttcgctggattcccagtatccggcctgtggcttcgttgcaccaacgaggaactgatcgagcagcacgcagccaaggtatatggcaaggcatctgttggcgctcctccaatgtctgttcctcaccttgacacccgcgttatcgagggtgaaaagggtctgctctttggaccttacggtggctggacccctaagttcttgaaggaaggctcctacctggacctgttcaagtccatccgcccagacaacattccttcctaccttggcgttgctgctcaggaatttgatctgaccaagtaccttgtcactgaagttctcaaggaccaggacaagcgtatggatgctcttcgcgagtacatgccagaggcacaaaacggcgattgggagaccatcgttgccggacagcgtgttcaggttattaagcctgcaggattccctaagttcggttccctggaattcggcaccaccttgatcaacaactccgaaggcaccatcgccggattgctcggtgcttcccctggagcatccatcgcaccttccgcaatgatcgagctgcttgagcgttgcttcggtgaccgcatgatcgagtggggcgacaagctgaaggacatgatcccttcctacggcaagaagcttgcttccgagccagcactgtttgagcagcagtgggcacgcacccagaagaccctgaagcttgaggaagcctaa

SEQ ID NO: 3 - protein, 500 aa, Corynebacterium glutamicum
MSDSPKNAPRITDEADVVLIGAGIMSSTLGAMLRQLEPSWTQIVFERLDGPAQESSSPWNNAGTGHSALCELNYTPEVKGKVEIAKAVGINEKFQVSRQFWSHLVEEGVLADPKEFINPVPHVSFGQGADQVAYIKARYEALKDHPLFQGMTYADDEATFTEKLPLMAKGRDFSDPVAISWIDEGTDINYGAQTKQYLDASEVEGTEIRYGHEVKSIKADGAKWIVTVKNVHTGDTKTIKANFVFVGAGGYALDLLRSAGIPQVKGFAGFPVSGLWLRCTNEELIEQHAAKVYGKASVGAPPMSVPHLDTRVIEGEKGLLFGPYGGWTPKFLKEGSYLDLFKSIRPDNIPSYLGVAAQEFDLTKYLVTEVLKDQDKRMDALREYMPEAQNGDWETIVAGQRVQVIKPAGFPKFGSLEFGTTLINNSEGTIAGLLGASPGASIAPSAMIELLERCFGDRMIEWGDKLKDMIPSYGKKLASEPALFEQQWARTQKTLKLEEA

SEQ ID NO: 4 - protein, 500 aa, Artificial Sequence
  Synthesized
MSDSPKNAPRITDEADVVLIGAGIMSSTLGAMLRQLEPSWTQIVFERLDGPAQESSSPWNNAGTGHSALCELNYTPEVKGKVEIAKAVGINEKFQVSRQFWSHLVEEGVLADSKEFINPVPHVSFGQGADQVAYIKARYEALKDHPLFQGMTYADDEATFTEKLPLMAKGRDFSDPVAISWIDEGTDINYGAQTKQYLDASEVEGTEIRYGHEVKSIKADGAKWIVTVKNVHTGDTKTIKANFVFVGAGGYALDLLRSAGIPQVKGFAGFPVSGLWLRCTNEELIEQHAAKVYGKASVGAPPMSVPHLDTRVIEGEKGLLFGPYGGWTPKFLKEGSYLDLFKSIRPDNIPSYLGVAAQEFDLTKYLVTEVLKDQDKRMDALREYMPEAQNGDWETIVAGQRVQVIKPAGFPKFGSLEFGTTLINNSEGTIAGLLGASPGASIAPSAMIELLERCFGDRMIEWGDKLKDMIPSYGKKLASEPALFEQQWARTQKTLKLEEA

SEQ ID NO: 5 - DNA, 56 bp, Artificial Sequence
  Synthesized
cagtgccaagcttgcatgcctgcaggtcgactctagaaggaatgttgtctgggcgg

SEQ ID NO: 6 - DNA, 30 bp, Artificial Sequence
  Synthesized
ggcgtgctggctgattctaaggaattcatc

SEQ ID NO: 7 - DNA, 30 bp, Artificial Sequence
  Synthesized
gatgaattccttagaatcagccagcacgcc

SEQ ID NO: 8 - DNA, 58 bp, Artificial Sequence
  Synthesized
cagctatgaccatgattacgaattcgagctcggtacccgataggtcgattgttggtgt

SEQ ID NO: 9 - DNA, 20 bp, Artificial Sequence
  Synthesized
catcaaaggcagcttctcgg

SEQ ID NO: 10 - DNA, 20 bp, Artificial Sequence
  Synthesized
actacaccccagaggttaag

SEQ ID NO: 11 - DNA, 56 bp, Artificial Sequence
  Synthesized
cagtgccaagcttgcatgcctgcaggtcgactctaggacccgcttgccatacgaag

SEQ ID NO: 12 - DNA, 41 bp, Artificial Sequence
  Synthesized
ctgaagcttgaggaagcctaaatctactcatctgaagaatc

SEQ ID NO: 13 - DNA, 41 bp, Artificial Sequence
  Synthesized
gattcttcagatgagtagatttaggcttcctcaagcttcag

SEQ ID NO: 14 - DNA, 39 bp, Artificial Sequence
  Synthesized
caaaccagagtgcccacgaaatgtataacgataggtcga

SEQ ID NO: 15 - DNA, 39 bp, Artificial Sequence
  Synthesized
tcgacctatcgttatacatttcgtgggcactctggtttg

SEQ ID NO: 16 - DNA, 58 bp, Artificial Sequence
  Synthesized
cagctatgaccatgattacgaattcgagctcggtaccccataagaaacaaccacttcc

SEQ ID NO: 17 - DNA, 20 bp, Artificial Sequence
  Synthesized
gtccaaggtgacggccgcac

SEQ ID NO: 18 - DNA, 20 bp, Artificial Sequence
  Synthesized
tgacttctctgatccagtag

SEQ ID NO: 19 - DNA, 20 bp, Artificial Sequence
  Synthesized
gtactgcttggtctgagcac

SEQ ID NO: 20 - DNA, 20 bp, Artificial Sequence
  Synthesized
atattcggcccagcagcagc

SEQ ID NO: 21 - DNA, 57 bp, Artificial Sequence
  Synthesized
gcttgcatgcctgcaggtcgactctagaggatccccttaggcttcctcaagcttcag

SEQ ID NO: 22 - DNA, 53 bp, Artificial Sequence
  Synthesized
atcaggctgaaaatcttctctcatccgccaaaacatgtataacgataggtcga

SEQ ID NO: 23 - DNA, 56 bp, Artificial Sequence
  Synthesized
cagtgccaagcttgcatgcctgcaggtcgactctaggcctgactgattttgggctg

SEQ ID NO: 24 - DNA, 40 bp, Artificial Sequence
  Synthesized
gagataaaaggaagttgaacatcttctaactgctttcttt

SEQ ID NO: 25 - DNA, 40 bp, Artificial Sequence
  Synthesized
aaagaaagcagttagaagatgttcaacttccttttatctc

SEQ ID NO: 26 - DNA, 58 bp, Artificial Sequence
  Synthesized
cagctatgaccatgattacgaattcgagctcggtacccagatgacctcggcagcagct

SEQ ID NO: 27 - DNA, 20 bp, Artificial Sequence
  Synthesized
gcctgactgattttgggctg

SEQ ID NO: 28 - DNA, 20 bp, Artificial Sequence
  Synthesized
agatgacctcggcagcagct

SEQ ID NO: 29 - DNA, 1504 bp, Artificial Sequence
  Synthesized
cagtgccaagcttgcatgcctgcaggtcgactctagaaggaatgttgtctgggcggatggacttgaacaggtccaggtaggagccttccttcaagaacttaggggtccagccaccgtaaggtccaaagagcagacccttttcaccctcgataacgcgggtgtcaaggtgaggaacagacattggaggagcgccaacagatgccttgccatataccttggctgcgtgctgctcgatcagttcctcgttggtgcaacgaagccacaggccggatactgggaatccagcgaagcccttgacctgtgggatgcctgcgctgcgaagcagatccagtgcgtacccgcctgcgccgacgaacacgaagtttgccttgatggtcttggtgtcgccagtgtgtacgttcttgacggtcacgatccactttgcgccatcagccttgatgctcttgacttcgtggccatagcggatttcagtgccttcaacttcagatgcatccaggtactgcttggtctgagcaccgtagttgatgtcggtgccttcatcgatccaagagattgctactggatcagagaagtcacggccctttgccatcaaaggcagcttctcggtgaaggtagcttcatcgtcagcgtaggtcatgccctggaagagtgggtgatccttcaaagcttcgtagcgagccttgatgtatgcaacctggtctgcgccctggccgaaagatacgtgaggaacagggttgatgaattccttagaatcagccagcacgccctcttcaacgaggtgagaccagaactgacgggaaacctggaacttctcgttgattcctacagccttggcaatttcaaccttgcccttaacctctggggtgtagttcagctcgcatagagcagagtggccggttcctgcattgttccacggggaggacgactcttgtgccggtccatccaaacgctcgaagacgatctgagtccagcttggctccagctgacgcagcattgcacccagcgtggagctcatgataccggcaccaatgagaactacatctgcctcatcggtaatcctcggtgcgttcttcggggaatctgacatgttcaacttccttttatctccgcgagttctctgccgaacaccaacacaaggcgtcatctcataaatgatcgccagcacccgaatgcaagtgttggccatatttttgactgacgcgtggggcgttacccttcttgtttcttacaagaaagcgtgggtacacattgtccgtaaatatagagtgtacgcctgccacctcgagctgaataaacaagcacgggatattcccctttctcatgcgaattcctcccccgtgctaccccctcccccaatttgcaaagttagtaaatgtgaaattcgcaaacatgagtagtatcgcggaagtttcaccacgtgaacctttcagtcggctcgcgcacaccacaccaacaatcgacctatcgggtaccgagctcgaattcgtaatcatggtcatagctg

SEQ ID NO: 30 - DNA, 3445 bp, Artificial Sequence
  Synthesized
cagtgccaagcttgcatgcctgcaggtcgactctaggacccgcttgccatacgaagtcctggagaagatctccacccgcatcaccaacgaagttccagacgtaaaccgcgtggttttggacgtaacctccaagccaccaggaaccatcgaatgggagtaggccttaaatgagccttcgttaagcggcaatcaccttatcggtgattgccgctttcccatttctccgggttttctggaactttttgggcgtatgctgggaatgatcttattattttgatttcagaaagcaggagagaccagatgagcgaaatccttgaaacctactgggcaccccacttcggaaacaccgatgaagccgcagcactcgtttcatacttggcacaagcttccggtgatcctattgaggttcacaccctgttcggggatttaggtttagacggactctctggaaactacaccgacactgagatcgacggctacggcgacgcattcctgctggttgcagcactagcagtgttgatggctgaaaacaaagcatccggcggcgtgaatctgggtgaagttgggggagctgataaatcgatccggctgcatgttgaatccaaggaaaacacccagatcaacaccgcattgaagtactttgcgctttccccagaagaccacgcagcggcagatcgcttcgatgaggatgacctgtctgagcttgccaacttgagtgaagagctgcgcggacagctggactaattgctgcccgtttaaggagtccgattcttcagatgagtagatttaggcttcctcaagcttcagggtcttctgggtgcgtgcccactgctgctcaaacagtgctggctcggaagcaagcttcttgccgtaggaagggatcatgtccttcagcttgtcgccccactcgatcatgcggtcaccgaagcaacgctcaagcagctcgatcattgcggaaggtgcgatggatgctccaggggaagcaccgagcaatccggcgatggtgccttcggagttgttgatcaaggtggtgccgaattccagggaaccgaacttagggaatcctgcaggcttaataacctgaacacgctgtccggcaacgatggtctcccaatcgccgttttgtgcctctggcatgtactcgcgaagagcatccatacgcttgtcctggtccttgagaacttcagtgacaaggtacttggtcagatcaaattcctgagcagcaacgccaaggtaggaaggaatgttgtctgggcggatggacttgaacaggtccaggtaggagccttccttcaagaacttaggggtccagccaccgtaaggtccaaagagcagacccttttcaccctcgataacgcgggtgtcaaggtgaggaacagacattggaggagcgccaacagatgccttgccatataccttggctgcgtgctgctcgatcagttcctcgttggtgcaacgaagccacaggccggatactgggaatccagcgaagcccttgacctgtgggatgcctgcgctgcgaagcagatccagtgcgtacccgcctgcgccgacgaacacgaagtttgccttgatggtcttggtgtcgccagtgtgtacgttcttgacggtcacgatccactttgcgccatcagccttgatgctcttgacttcgtggccatagcggatttcagtgccttcaacttcagatgcatccaggtactgcttggtctgagcaccgtagttgatgtcggtgccttcatcgatccaagagattgctactggatcagagaagtcacggccctttgccatcaaaggcagcttctcggtgaaggtagcttcatcgtcagcgtaggtcatgccctggaagagtgggtgatccttcaaagcttcgtagcgagccttgatgtatgcaacctggtctgcgccctggccgaaagatacgtgaggaacagggttgatgaattccttaggatcagccagcacgccctcttcaacgaggtgagaccagaactgacgggaaacctggaacttctcgttgattcctacagccttggcaatttcaaccttgcccttaacctctggggtgtagttcagctcgcatagagcagagtggccggttcctgcattgttccacggggaggacgactcttgtgccggtccatccaaacgctcgaagacgatctgagtccagcttggctccagctgacgcagcattgcacccagcgtggagctcatgataccggcaccaatgagaactacatctgcctcatcggtaatcctcggtgcgttcttcggggaatctgacatgttcaacttccttttatctccgcgagttctctgccgaacaccaacacaaggcgtcatctcataaatgatcgccagcacccgaatgcaagtgttggccatatttttgactgacgcgtggggcgttacccttcttgtttcttacaagaaagcgtgggtacacattgtccgtaaatatagagtgtacgcctgccacctcgagctgaataaacaagcacgggatattcccctttctcatgcgaattcctcccccgtgctaccccctcccccaatttgcaaagttagtaaatgtgaaattcgcaaacatgagtagtatcgcggaagtttcaccacgtgaacctttcagtcggctcgcgcacaccacaccaacaatcgacctatcgttatacatttcgtgggcactctggtttggttaccaggatgggttagtcattctgatcagcgaattccacgttcacatcgccaattccagagttcacaaccagattcagcattggaccttctagatcagcattgtgggcggtgagatctccaacatcacagcgcgctgtgcccacaccggcggtacaacttaggctcacgggcacatcatcgggcagggtgaccatgacttcgccgatccctgaggtgatttggatgttttgttcctgatccaattgggtgaggtggctgaaatcgaggttcatttcacccacgccagaggtgtagctgctgaggagttcatcgttggtggggatgagattgacatcgccgattccagggtcgtcttcaaagtagatgggatcgatatttgaaataaacaggcctgcgagggcgctcatgacaactccggtaccaactacaccgccgacaatccatggccacacatggcgctttttctgaggcttttgtggagggacttgtacatcccaggtgttgtattggttttgggcaagtggatcccaatgaggcgcttcgggggtttgttgcgcgaagggtgcatagtagccctcaacgggggtgatagtgcttagatctggttggggttgtgggtagagatcttcgtttttcatggtggcatcctcagaaacagtgaattcagtggtgagtagtccgcggggtggaagtggttgtttcttatggggtaccgagctcgaattcgtaatcatggtcatagctg

SEQ ID NO: 31 - DNA, 3445 bp, Artificial Sequence
  Synthesized
cagtgccaagcttgcatgcctgcaggtcgactctaggacccgcttgccatacgaagtcctggagaagatctccacccgcatcaccaacgaagttccagacgtaaaccgcgtggttttggacgtaacctccaagccaccaggaaccatcgaatgggagtaggccttaaatgagccttcgttaagcggcaatcaccttatcggtgattgccgctttcccatttctccgggttttctggaactttttgggcgtatgctgggaatgatcttattattttgatttcagaaagcaggagagaccagatgagcgaaatccttgaaacctactgggcaccccacttcggaaacaccgatgaagccgcagcactcgtttcatacttggcacaagcttccggtgatcctattgaggttcacaccctgttcggggatttaggtttagacggactctctggaaactacaccgacactgagatcgacggctacggcgacgcattcctgctggttgcagcactagcagtgttgatggctgaaaacaaagcatccggcggcgtgaatctgggtgaagttgggggagctgataaatcgatccggctgcatgttgaatccaaggaaaacacccagatcaacaccgcattgaagtactttgcgctttccccagaagaccacgcagcggcagatcgcttcgatgaggatgacctgtctgagcttgccaacttgagtgaagagctgcgcggacagctggactaattgctgcccgtttaaggagtccgattcttcagatgagtagatttaggcttcctcaagcttcagggtcttctgggtgcgtgcccactgctgctcaaacagtgctggctcggaagcaagcttcttgccgtaggaagggatcatgtccttcagcttgtcgccccactcgatcatgcggtcaccgaagcaacgctcaagcagctcgatcattgcggaaggtgcgatggatgctccaggggaagcaccgagcaatccggcgatggtgccttcggagttgttgatcaaggtggtgccgaattccagggaaccgaacttagggaatcctgcaggcttaataacctgaacacgctgtccggcaacgatggtctcccaatcgccgttttgtgcctctggcatgtactcgcgaagagcatccatacgcttgtcctggtccttgagaacttcagtgacaaggtacttggtcagatcaaattcctgagcagcaacgccaaggtaggaaggaatgttgtctgggcggatggacttgaacaggtccaggtaggagccttccttcaagaacttaggggtccagccaccgtaaggtccaaagagcagacccttttcaccctcgataacgcgggtgtcaaggtgaggaacagacattggaggagcgccaacagatgccttgccatataccttggctgcgtgctgctcgatcagttcctcgttggtgcaacgaagccacaggccggatactgggaatccagcgaagcccttgacctgtgggatgcctgcgctgcgaagcagatccagtgcgtacccgcctgcgccgacgaacacgaagtttgccttgatggtcttggtgtcgccagtgtgtacgttcttgacggtcacgatccactttgcgccatcagccttgatgctcttgacttcgtggccatagcggatttcagtgccttcaacttcagatgcatccaggtactgcttggtctgagcaccgtagttgatgtcggtgccttcatcgatccaagagattgctactggatcagagaagtcacggccctttgccatcaaaggcagcttctcggtgaaggtagcttcatcgtcagcgtaggtcatgccctggaagagtgggtgatccttcaaagcttcgtagcgagccttgatgtatgcaacctggtctgcgccctggccgaaagatacgtgaggaacagggttgatgaattccttagaatcagccagcacgccctcttcaacgaggtgagaccagaactgacgggaaacctggaacttctcgttgattcctacagccttggcaatttcaaccttgcccttaacctctggggtgtagttcagctcgcatagagcagagtggccggttcctgcattgttccacggggaggacgactcttgtgccggtccatccaaacgctcgaagacgatctgagtccagcttggctccagctgacgcagcattgcacccagcgtggagctcatgataccggcaccaatgagaactacatctgcctcatcggtaatcctcggtgcgttcttcggggaatctgacatgttcaacttccttttatctccgcgagttctctgccgaacaccaacacaaggcgtcatctcataaatgatcgccagcacccgaatgcaagtgttggccatatttttgactgacgcgtggggcgttacccttcttgtttcttacaagaaagcgtgggtacacattgtccgtaaatatagagtgtacgcctgccacctcgagctgaataaacaagcacgggatattcccctttctcatgcgaattcctcccccgtgctaccccctcccccaatttgcaaagttagtaaatgtgaaattcgcaaacatgagtagtatcgcggaagtttcaccacgtgaacctttcagtcggctcgcgcacaccacaccaacaatcgacctatcgttatacatttcgtgggcactctggtttggttaccaggatgggttagtcattctgatcagcgaattccacgttcacatcgccaattccagagttcacaaccagattcagcattggaccttctagatcagcattgtgggcggtgagatctccaacatcacagcgcgctgtgcccacaccggcggtacaacttaggctcacgggcacatcatcgggcagggtgaccatgacttcgccgatccctgaggtgatttggatgttttgttcctgatccaattgggtgaggtggctgaaatcgaggttcatttcacccacgccagaggtgtagctgctgaggagttcatcgttggtggggatgagattgacatcgccgattccagggtcgtcttcaaagtagatgggatcgatatttgaaataaacaggcctgcgagggcgctcatgacaactccggtaccaactacaccgccgacaatccatggccacacatggcgctttttctgaggcttttgtggagggacttgtacatcccaggtgttgtattggttttgggcaagtggatcccaatgaggcgcttcgggggtttgttgcgcgaagggtgcatagtagccctcaacgggggtgatagtgcttagatctggttggggttgtgggtagagatcttcgtttttcatggtggcatcctcagaaacagtgaattcagtggtgagtagtccgcggggtggaagtggttgtttcttatggggtaccgagctcgaattcgtaatcatggtcatagctg

SEQ ID NO: 32 - DNA, 1961 bp, Artificial Sequence
  Synthesized
gcttgcatgcctgcaggtcgactctagaggatccccttaggcttcctcaagcttcagggtcttctgggtgcgtgcccactgctgctcaaacagtgctggctcggaagcaagcttcttgccgtaggaagggatcatgtccttcagcttgtcgccccactcgatcatgcggtcaccgaagcaacgctcaagcagctcgatcattgcggaaggtgcgatggatgctccaggggaagcaccgagcaatccggcgatggtgccttcggagttgttgatcaaggtggtgccgaattccagggaaccgaacttagggaatcctgcaggcttaataacctgaacacgctgtccggcaacgatggtctcccaatcgccgttttgtgcctctggcatgtactcgcgaagagcatccatacgcttgtcctggtccttgagaacttcagtgacaaggtacttggtcagatcaaattcctgagcagcaacgccaaggtaggaaggaatgttgtctgggcggatggacttgaacaggtccaggtaggagccttccttcaagaacttaggggtccagccaccgtaaggtccaaagagcagacccttttcaccctcgataacgcgggtgtcaaggtgaggaacagacattggaggagcgccaacagatgccttgccatataccttggctgcgtgctgctcgatcagttcctcgttggtgcaacgaagccacaggccggatactgggaatccagcgaagcccttgacctgtgggatgcctgcgctgcgaagcagatccagtgcgtacccgcctgcgccgacgaacacgaagtttgccttgatggtcttggtgtcgccagtgtgtacgttcttgacggtcacgatccactttgcgccatcagccttgatgctcttgacttcgtggccatagcggatttcagtgccttcaacttcagatgcatccaggtactgcttggtctgagcaccgtagttgatgtcggtgccttcatcgatccaagagattgctactggatcagagaagtcacggccctttgccatcaaaggcagcttctcggtgaaggtagcttcatcgtcagcgtaggtcatgccctggaagagtgggtgatccttcaaagcttcgtagcgagccttgatgtatgcaacctggtctgcgccctggccgaaagatacgtgaggaacagggttgatgaattccttaggatcagccagcacgccctcttcaacgaggtgagaccagaactgacgggaaacctggaacttctcgttgattcctacagccttggcaatttcaaccttgcccttaacctctggggtgtagttcagctcgcatagagcagagtggccggttcctgcattgttccacggggaggacgactcttgtgccggtccatccaaacgctcgaagacgatctgagtccagcttggctccagctgacgcagcattgcacccagcgtggagctcatgataccggcaccaatgagaactacatctgcctcatcggtaatcctcggtgcgttcttcggggaatctgacatgttcaacttccttttatctccgcgagttctctgccgaacaccaacacaaggcgtcatctcataaatgatcgccagcacccgaatgcaagtgttggccatatttttgactgacgcgtggggcgttacccttcttgtttcttacaagaaagcgtgggtacacattgtccgtaaatatagagtgtacgcctgccacctcgagctgaataaacaagcacgggatattcccctttctcatgcgaattcctcccccgtgctaccccctcccccaatttgcaaagttagtaaatgtgaaattcgcaaacatgagtagtatcgcggaagtttcaccacgtgaacctttcagtcggctcgcgcacaccacaccaacaatcgacctatcgttatacatgttttggcggatgagagaagattttcagcctgat

SEQ ID NO: 33 - DNA, 1961 bp, Artificial Sequence
  Synthesized
gcttgcatgcctgcaggtcgactctagaggatccccttaggcttcctcaagcttcagggtcttctgggtgcgtgcccactgctgctcaaacagtgctggctcggaagcaagcttcttgccgtaggaagggatcatgtccttcagcttgtcgccccactcgatcatgcggtcaccgaagcaacgctcaagcagctcgatcattgcggaaggtgcgatggatgctccaggggaagcaccgagcaatccggcgatggtgccttcggagttgttgatcaaggtggtgccgaattccagggaaccgaacttagggaatcctgcaggcttaataacctgaacacgctgtccggcaacgatggtctcccaatcgccgttttgtgcctctggcatgtactcgcgaagagcatccatacgcttgtcctggtccttgagaacttcagtgacaaggtacttggtcagatcaaattcctgagcagcaacgccaaggtaggaaggaatgttgtctgggcggatggacttgaacaggtccaggtaggagccttccttcaagaacttaggggtccagccaccgtaaggtccaaagagcagacccttttcaccctcgataacgcgggtgtcaaggtgaggaacagacattggaggagcgccaacagatgccttgccatataccttggctgcgtgctgctcgatcagttcctcgttggtgcaacgaagccacaggccggatactgggaatccagcgaagcccttgacctgtgggatgcctgcgctgcgaagcagatccagtgcgtacccgcctgcgccgacgaacacgaagtttgccttgatggtcttggtgtcgccagtgtgtacgttcttgacggtcacgatccactttgcgccatcagccttgatgctcttgacttcgtggccatagcggatttcagtgccttcaacttcagatgcatccaggtactgcttggtctgagcaccgtagttgatgtcggtgccttcatcgatccaagagattgctactggatcagagaagtcacggccctttgccatcaaaggcagcttctcggtgaaggtagcttcatcgtcagcgtaggtcatgccctggaagagtgggtgatccttcaaagcttcgtagcgagccttgatgtatgcaacctggtctgcgccctggccgaaagatacgtgaggaacagggttgatgaattccttagaatcagccagcacgccctcttcaacgaggtgagaccagaactgacgggaaacctggaacttctcgttgattcctacagccttggcaatttcaaccttgcccttaacctctggggtgtagttcagctcgcatagagcagagtggccggttcctgcattgttccacggggaggacgactcttgtgccggtccatccaaacgctcgaagacgatctgagtccagcttggctccagctgacgcagcattgcacccagcgtggagctcatgataccggcaccaatgagaactacatctgcctcatcggtaatcctcggtgcgttcttcggggaatctgacatgttcaacttccttttatctccgcgagttctctgccgaacaccaacacaaggcgtcatctcataaatgatcgccagcacccgaatgcaagtgttggccatatttttgactgacgcgtggggcgttacccttcttgtttcttacaagaaagcgtgggtacacattgtccgtaaatatagagtgtacgcctgccacctcgagctgaataaacaagcacgggatattcccctttctcatgcgaattcctcccccgtgctaccccctcccccaatttgcaaagttagtaaatgtgaaattcgcaaacatgagtagtatcgcggaagtttcaccacgtgaacctttcagtcggctcgcgcacaccacaccaacaatcgacctatcgttatacatgttttggcggatgagagaagattttcagcctgat